European Patent Specification EP 3 585 886 B1, published November 22, 2023. Title: LARGE SCALE SYNTHESIS OF MESSENGER RNA. Applicant: TRANSLATE BIO INC. The sequence listing filed with the application follows.

SEQUENCE LISTING (13 sequences)

SEQ ID NO: 1 - protein, 874 aa, Bacteriophage SP6
MQDLHAIQLQLEEEMFNGGIRRFEADQQRQIAAGSESDTAWNRRLLSELIAPMAEGIQAYKEEYEGKKGRAPRALAFLQCVENEVAAYITMKVVMDMLNTDATLQAIAMSVAERIEDQVRFSKLEGHAAKYFEKVKKSLKASRTKSYRHAHNVAVVAEKSVAEKDADFDRWEAWPKETQLQIGTTLLEILEGSVFYNGEPVFMRAMRTYGGKTIYYLQTSESVGQWISAFKEHVAQLSPAYAPCVIPPRPWRTPFNGGFHTEKVASRIRLVKGNREHVRKLTQKQMPKVYKAINALQNTQWQINKDVLAVIEEVIRLDLGYGVPSFKPLIDKENKPANPVPVEFQHLRGRELKEMLSPEQWQQFINWKGECARLYTAETKRGSKSAAVVRMVGQARKYSAFESIYFVYAMDSRSRVYVQSSTLSPQSNDLGKALLRFTEGRPVNGVEALKWFCINGANLWGWDKKTFDVRVSNVLDEEFQDMCRDIAADPLTFTQWAKADAPYEFLAWCFEYAQYLDLVDEGRADEFRTHLPVHQDGSCSGIQHYSAMLRDEVGAKAVNLKPSDAPQDIYGAVAQVVIKKNALYMDADDATTFTSGSVTLSGTELRAMASAWDSIGITRSLTKKPVMTLPYGSTRLTCRESVIDYIVDLEEKEAQKAVAEGRTANKVHPFEDDRQDYLTPGAAYNYMTALIWPSISEVVKAPIVAMKMIRQLARFAAKRNEGLMYTLPTGFILEQKIMATEMLRVRTCLMGDIKMSLQVETDIVDEAAMMGAAAPNFVHGHDASHLILTVCELVDKGVTSIAVIHDSFGTHADNTLTLRVALKGQMVAMYIDGNALQKLLEEHEVRWMVDTGIEVPEQGEFDLNEIMDSEYVFA

SEQ ID NO: 2 - DNA, 2625 bp, Bacteriophage SP6
atgcaagatttacacgctatccagcttcaattagaagaagagatgtttaatggtggcattcgtcgcttcgaagcagatcaacaacgccagattgcagcaggtagcgagagcgacacagcatggaaccgccgcctgttgtcagaacttattgcacctatggctgaaggcattcaggcttataaagaagagtacgaaggtaagaaaggtcgtgcacctcgcgcattggctttcttacaatgtgtagaaaatgaagttgcagcatacatcactatgaaagttgttatggatatgctgaatacggatgctacccttcaggctattgcaatgagtgtagcagaacgcattgaagaccaagtgcgcttttctaagctagaaggtcacgccgctaaatactttgagaaggttaagaagtcactcaaggctagccgtactaagtcatatcgtcacgctcataacgtagctgtagttgctgaaaaatcagttgcagaaaaggacgcggactttgaccgttgggaggcgtggccaaaagaaactcaattgcagattggtactaccttgcttgaaatcttagaaggtagcgttttctataatggtgaacctgtatttatgcgtgctatgcgcacttatggcggaaagactatttactacttacaaacttctgaaagtgtaggccagtggattagcgcattcaaagagcacgtagcgcaattaagcccagcttatgccccttgcgtaatccctcctcgtccttggagaactccatttaatggagggttccatactgagaaggtagctagccgtatccgtcttgtaaaaggtaaccgtgagcatgtacgcaagttgactcaaaagcaaatgccaaaggtttataaggctatcaacgcattacaaaatacacaatggcaaatcaacaaggatgtattagcagttattgaagaagtaatccgcttagaccttggttatggtgtaccttccttcaagccactgattgacaaggagaacaagccagctaacccggtacctgttgaattccaacacctgcgcggtcgtgaactgaaagagatgctatcacctgagcagtggcaacaattcattaactggaaaggcgaatgcgcgcgcctatataccgcagaaactaagcgcggttcaaagtccgccgccgttgttcgcatggtaggacaggcccgtaaatatagcgcctttgaatccatttacttcgtgtacgcaatggatagccgcagccgtgtctatgtgcaatctagcacgctctctccgcagtctaacgacttaggtaaggcattactccgctttaccgagggacgccctgtgaatggcgtagaagcgcttaaatggttctgcatcaatggtgctaacctttggggatgggacaagaaaacttttgatgtgcgcgtgtctaacgtattagatgaggaattccaagatatgtgtcgagacatcgccgcagaccctctcacattcacccaatgggctaaagctgatgcaccttatgaattcctcgcttggtgctttgagtatgctcaataccttgatttggtggatgaaggaagggccgacgaattccgcactcacctaccagtacatcaggacgggtcttgttcaggcattcagcactatagtgctatgcttcgcgacgaagtaggggccaaagctgttaacctgaaaccctccgatgcaccgcaggatatctatggggcggtggcgcaagtggttatcaagaagaatgcgctatatatggatgcggacgatgcaaccacgtttacttctggtagcgtcacgctgtccggtacagaactgcgagcaatggctagcgcatgggatagtattggtattacccgtagcttaaccaaaaagcccgtgatgaccttgccatatggttctactcgcttaacttgccgtgaatctgtgattgattacatcgtagacttagaggaaaaagaggcgcagaaggcagtagcagaagggcggacggcaaacaaggtacatccttttgaagacgatcgtcaagattacttgactccgggcgcagcttacaactacatgacggcactaatctggccttctatttctgaagtagttaaggcaccgatagtagctatgaagatgatacgccagcttgcacgctttgcagcgaaacgtaatgaaggcctgatgtacaccctgcctactggcttcatcttagaacagaagatcatggcaaccgagatgctacgcgtgcgtacctgtctgatgggtgatatcaagatgtcccttcaggttgaaacggatatcgtagatgaagccgctatgatgggagcagcagcacctaatttcgtacacggtcatgacgcaagtcaccttatccttaccgtatgtgaattggtagacaagggcgtaactagtatcgctgtaatccacgactcttttggtactcatgcagacaacaccctcactcttagagtggcacttaaagggcagatggttgcaatgtatattgatggtaatgcgcttcagaaactactggaggagcatgaagtgcgctggatggttgatacaggtatcgaagtacctgagcaaggggagttcgaccttaacgaaatcatggattctgaatacgtatttgcctaa

SEQ ID NO: 3 - DNA, 18 bp, Bacteriophage SP6
atttaggtgacactatag

SEQ ID NO: 4 - DNA, 23 bp, Artificial Sequence
  Synthetic oligonucleotide
atttaggggacactatagaagag

SEQ ID NO: 5 - DNA, 22 bp, Artificial Sequence
  Synthetic oligonucleotide
atttaggggacactatagaagg

SEQ ID NO: 6 - DNA, 23 bp, Artificial Sequence
  Synthetic oligonucleotide
atttaggggacactatagaaggg

SEQ ID NO: 7 - DNA, 20 bp, Artificial Sequence
  Synthetic oligonucleotide
atttaggtgacactatagaa

SEQ ID NO: 8 - DNA, 22 bp, Artificial Sequence
  Synthetic oligonucleotide
atttaggtgacactatagaaga

SEQ ID NO: 9 - DNA, 23 bp, Artificial Sequence
  9
atttaggtgacactatagaagag

SEQ ID NO: 10 - DNA, 22 bp, Artificial Sequence
  Synthetic oligonucleotide
atttaggtgacactatagaagg

SEQ ID NO: 11 - DNA, 23 bp, Artificial Sequence
  Synthetic oligonucleotide
atttaggtgacactatagaaggg

SEQ ID NO: 12 - DNA, 23 bp, Artificial Sequence
  Synthetic oligonucleotide
  misc_feature (22)..(22): n is a, c, g, or t
atttaggtgacactatagaagng

SEQ ID NO: 13 - DNA, 24 bp, Artificial Sequence
  Synthetic oligonucleotide
catacgatttaggtgacactatag